European Patent Specification EP 3 564 368 B1, published March 26, 2025. Title: Mutant Nitrile Hydratase, Nucleic Acid Encoding the Mutant Nitrile Hydratase, Expression Vector and Transformant Containing the Nucleic Acid, Production Method for Muntant Nitrile Hydratase, and Production Method for Amide Compound. Applicant: MITSUI CHEMICALS, INC. The sequence listing filed with the application follows.

SEQUENCE LISTING (75 sequences)

SEQ ID NO: 1 - protein, 205 aa, Pseudonocardia thermophila
MTENILRKSDEEIQKEITARVKALESMLIEQGILTTSMIDRMAEIYENEVGPHLGAKVVVKAWTDPEFKKRLLADGTEACKELGIGGLQGEDMMWVENTDEVHHVVVCTLCSCYPWPVLGLPPNWFKEPQYRSRVVREPRQLLKEEFGFEVPPSKEIKVWDSSSEMRFVVLPQRPAGTDGWSEEELATLVTRESMIGVEPAKAVA

SEQ ID NO: 2 - protein, 233 aa, Pseudonocardia thermophila
MNGVYDVGGTDGLGPINRPADEPVFRAEWEKVAFAMFPATFRAGFMGLDEFRFGIEQMNPAEYLESPYYWHWIRTYIHHGVRTGKIDLEELERRTQYYRENPDAPLPEHEQKPELIEFVNQAVYGGLPASREVDRPPKFKEGDVVRFSTASPKGHARRARYVRGKTGTVVKHHGAYIYPDTAGNGLGECPEHLYTVRFTAQELWGPEGDPNSSVYYDCWEPYIELVDTKAAAA

SEQ ID NO: 3 - DNA, 618 bp, Pseudonocardia thermophila
atgaccgagaacatcctgcgcaagtcggacgaggagatccagaaggagatcacggcgcgggtcaaggccctggagtcgatgctcatcgaacagggcatcctcaccacgtcgatgatcgaccggatggccgagatctacgagaacgaggtcggcccgcacctcggcgcgaaggtcgtcgtgaaggcctggaccgacccggagttcaagaagcgtctgctcgccgacggcaccgaggcctgcaaggagctcggcatcggcggcctgcagggcgaggacatgatgtgggtggagaacaccgacgaggtccaccacgtcgtcgtgtgcacgctctgctcctgctacccgtggccggtgctggggctgccgccgaactggttcaaggagccgcagtaccgctcccgcgtggtgcgtgagccccggcagctgctcaaggaggagttcggcttcgaggtcccgccgagcaaggagatcaaggtctgggactccagctccgagatgcgcttcgtcgtcctcccgcagcgccccgcgggcaccgacgggtggagcgaggaggagctcgccaccctcgtcacccgcgagtcgatgatcggcgtcgaaccggcgaaggcggtcgcgtga

SEQ ID NO: 4 - DNA, 702 bp, Pseudonocardia thermophila
atgaacggcgtgtacgacgtcggcggcaccgatgggctgggcccgatcaaccggcccgcggacgaaccggtcttccgcgccgagtgggagaaggtcgcgttcgcgatgttcccggcgacgttccgggccggcttcatgggcctggacgagttccggttcggcatcgagcagatgaacccggccgagtacctcgagtcgccgtactactggcactggatccgcacctacatccaccacggcgtccgcaccggcaagatcgatctcgaggagctggagcgccgcacgcagtactaccgggagaaccccgacgccccgctgcccgagcacgagcagaagccggagttgatcgagttcgtcaaccaggccgtctacggcgggctgcccgcaagccgggaggtcgaccgaccgcccaagttcaaggagggcgacgtggtgcggttctccaccgcgagcccgaagggccacgcccggcgcgcgcggtacgtgcgcggcaagaccgggacggtggtcaagcaccacggcgcgtacatctacccggacaccgccggcaacggcctgggcgagtgccccgagcacctctacaccgtccgcttcacggcccaggagctgtgggggccggaaggggacccgaactccagcgtctactacgactgctgggagccctacatcgagctcgtcgacacgaaggcggccgcggcatga

SEQ ID NO: 5 - DNA, 24 bp, Artificial
  Primer
cagggcgaggagatgatgtgggtg

SEQ ID NO: 6 - DNA, 21 bp, Artificial
  Primer
atcctcacctggtcgatgatc

SEQ ID NO: 7 - DNA, 21 bp, Artificial
  Primer
gtcgatgatcaaccggatggc

SEQ ID NO: 8 - DNA, 20 bp, Artificial
  Primer
accggatggtcgagatctac

SEQ ID NO: 9 - DNA, 21 bp, Artificial
  Primer
gagctgtgggtgccggaaggg

SEQ ID NO: 10 - DNA, 21 bp, Artificial
  Primer
ctgtgggggcaggaaggggac

SEQ ID NO: 11 - DNA, 21 bp, Artificial
  primer
ctccagcgtcaactacgactg

SEQ ID NO: 12 - DNA, 17 bp, Artificial
  Primer
gttttcccagtcacgac

SEQ ID NO: 13 - DNA, 17 bp, Artificial
  Primer
caggaaacagctatgac

SEQ ID NO: 14 - DNA, 20 bp, Artificial
  Primer
ggccagtgcctagcttacat

SEQ ID NO: 15 - DNA, 20 bp, Artificial
  Primer
gctgtgggtgcaggaagggg

SEQ ID NO: 16 - protein, 205 aa, Artificial
  Modified nitrile hydratase alpha-subunit
MTENILRKSDEEIQKEITARVKALESMLIEQGILTMSMIDRMAEIYENEVGPHLGAKVVVKAWTDPEFKKRLLADGTEACKELGIGGLQGEDMMWVENTDEVHHVVVCTLCSCYPWPVLGLPPNWFKEPQYRSRVVREPRQLLKEEFDFEVPPSKEIKVWDSSSEMRFVVLPQRPAGTDGWSEEELATLVTRESMIGVEPAKARA

SEQ ID NO: 17 - protein, 205 aa, Artificial
  Modified nitrile hydratase alpha-subunit
MTENILRKSDEEIQKEITARVKALESMLIEQGILTMSMIDRMAEIYENEVGPHLGAKVVVKAWTDPEFKKRLLADGTEACKELGIGGLQGEEMMWVENTDEVHHVVVCTLCSCYPWPVLGLPPNWFKEPQYRSRVVREPRQLLKEEFDFEVPPSKEIKVWDSSSEMRFVVLPQRPAGTDGWSEEELATLVTRESMIGVEPAKARA

SEQ ID NO: 18 - protein, 205 aa, Artificial
  Modified nitrile hydratase alpha-subunit
MTENITRKSDEEIQKEITVRVKALESMLIEQGILTTSMIDRMAEIYENEVGPHLGAKVVVKAWTDPEFKKRLLADGTEACKELGIGGLQGEDMMWVENTDEVHHVVVCTLCSCYPWPVLGLPPNWYKEPQYRSRVVREPRQLLKEEFGFEVPPSKEIKVWDSSSEMRFVVLPQRPAGTDGWSEEELATLVTRESMIGVEPAKAVA

SEQ ID NO: 19 - protein, 205 aa, Artificial
  Modified nitrile hydratase alpha-subunit
MTENITRKSDEEIQKEITVRVKALESMLIEQGILTTSMIDRMAEIYENEVGPHLGAKVVVKAWTDPEFKKRLLADGTEACKELGIGGLQGEDMIWVENTDEVHHVVVCTLCSCYPWPVLGLPPNWYKEPQYRSRVVREPRQLLKEEFGFEVPPSKEIKVWDSSSEMRFVVLPQRPAGTDGWSEEELATLVTRESMIGVEPAKAVA

SEQ ID NO: 20 - protein, 205 aa, Artificial
  Modified nitrile hydratase alpha-subunit
MTENIARKSDEEIQKEITVRVKALESMLIEQGILTTSMIDRMAEIYENEVGPHLGAKVVVKAWTDPEFKKRLLADGTEACKELGIGGLQGEDMMWVENTDEVHHVVVCTLCSCYPWPVLGLPPNWYKEPQYRSRVVREPRQLLKEEFGFEVPPSKEIKVWDSSSEMRFVVLPQRPAGTDGWSEEELATLVTRESMIGVEPAKAVA

SEQ ID NO: 21 - protein, 205 aa, Artificial
  Modified nitrile hydratase alpha-subunit
MTENILRKSDEEIQKEITVRVKALESMLIEQGILTTSMIDRMAEIYENEVGPHLGAKVVVKAWTDPEFKKHLLADGTEACKELGIGGLQGEDMMWVENTDEVHHVVVCTLCSCYPWPVLGLPPNWYKEPQYRSRVVREPRQLLKEEFGFEVPPSKEIKVWDSSSEMRFVVLPQRPAGTDGWSEEELATLVTRESMIGVEPAKAVA

SEQ ID NO: 22 - protein, 205 aa, Artificial
  Modified nitrile hydratase alpha-subunit
MTENILRKSDEELQKEITVRVKALESMLIEQGILTTSMIDRMAEIYENEVGPHLGAKVVVKAWTDPEFKKHLLADGTEACKELGIGGLQGEDMMWVENTDEVHHVVVCTLCSCYPWPVLGLPPNWYKEPQYRSRVVREPRQLLKEEFGFEVPPSKEIKVWDSSSEMRFVVLPQRPAGTDGWSEEELATLVTRESMIGVEPAKAVA

SEQ ID NO: 23 - protein, 205 aa, Artificial
  Modified nitrile hydratase alpha-subunit
MTENITRKSDEEIQKEITARVKALESMLIEQGILTMSMIDRMAEIYENEVGPHLGAKVVVKAWTDPEFKKRLLADGTEACKELGIGGLQGEDMMWVENTDEVHHVVVCTLCSCYPWPVLGLPPNWYKEPQYRSRVVREPRQLLKEEFGFEVPPSKEIKVWDSSSEMRFVVLPQRPAGTDGWSEEELATLVTRESMIGVEPAKAVA

SEQ ID NO: 24 - protein, 205 aa, Artificial
  Modified nitrile hydratase alpha-subunit
MTENITRKSDEEIQKEITARVKALESILIEQGILTMSMIDRMAEIYENEVGPHLGAKVVVKAWTDPEFKKRLLADGTEACKELGIGGLQGEDMMWVENTDEVHHVVVCTLCSCYPWPVLGLPPNWYKEPQYRSRVVREPRQLLKEEFGFEVPPSKEIKVWDSSSEMRFVVLPQRPAGTDGWSEEELATLVTRESMIGVEPAKAVA

SEQ ID NO: 25 - protein, 205 aa, Artificial
  Modified nitrile hydratase alpha-subunit
MTENILRKSDEEIQKEITARVKALESMLIEQGILTTSMIDRMAEIYENEVGPHLGAKVVVKAWTDPEFKKRLLADGTEACKELGIGGLQGEEMMWVENTDEVHHVVVCTLCSCYPWPVLGLPPNWFKEPQYRSRVVREPRQLLKEEFDFEVPPSKEIKVWDSSSEMRFVVLPQRPAGTDGWSEEELATLVTRESMIGVEPAKARA

SEQ ID NO: 26 - protein, 205 aa, Artificial
  Modified nitrile hydratase alpha-subunit
MTENILRKSDEELQKEITVRVKALESILIEQGILTTSMIDRMAEIYENEVGPHLGAKVVVKAWTDPEFKKHLLADGTEACKELGIGGLQGEDMMWVENTDEVHHVVVCTLCSCYPWPVLGLPPNWYKEPQYRSRVVREPRQLLKEEFGFEVPPSKEIKVWDSSSEMRFVVLPQRPAGTDGWSEEELATLVTRESMIGVEPAKAVA

SEQ ID NO: 27 - protein, 205 aa, Artificial
  Modified nitrile hydratase alpha-subunit
MTENILRKSDEELQKEITARVKALESILIEQGILTTSMIDRMAEIYENEVGPHLGAKVVVKAWTDPEFKKRLLADGTEACKELGIGGLQGEDMMWVENTDEVHHVVVCTLCSCYPWPVLGLPPNWFKEPQYRSRVVREPRQLLKEEFGFEVPPSKEIKVWDSSSEMRFVVLPQRPAGTDGWSEEELATLVTRESMIGVEPAKAVA

SEQ ID NO: 28 - protein, 205 aa, Artificial
  Modified nitrile hydratase alpha-subunit
MTENILRKSDEELQKEITARVKALESMLIEQGILTTSMIDRMAEIYENEVGPHLGAKVVVKAWTDPEFKKRLLADGTEACKELGIGGLQGEDMMWVENTDEVHHVVVCTLCSCYPWPVLGLPPNWFKEPQYRSRVVREPRQLLKEEFGFEVPPSKEIKVWDSSSEMRFVVLPQRPAGTDGWSEEELATLVTRESMIGVEPAKAVA

SEQ ID NO: 29 - protein, 205 aa, Artificial
  Modified nitrile hydratase alpha-subunit
MTENILRKSDEEIQKEITARVKALESMLIEQGILTTSMIDRMAEIYENEVGPHLGAKVVVKAWTDPEFKKRLLADGTEACKELGIGGLQGEDMMWVENTDEVHHVVVCTLCSCYPWPVLGLPPNWFKEPQYRSRVVREPRQLLKEEFGFEVPPSKEIKVWDSSSEMRFVVLPQRPAGTDGWSEEELATLVTRESMICVEPAKAVA

SEQ ID NO: 30 - protein, 205 aa, Artificial
  Modified nitrile hydratase alpha-subunit
MTENILRKSDEEIQKEITARVKALESMLIEQGILTTSMIDRMAEIYENEVGPHLGAKVVVKAWTDPEFKKRLLADGTEACKELGIGGLQGEEMMWVENTDEVHHVVVCTLCSCYPWPVLGLPPNWFKEPQYRSRVVREPRQLLKEEFGFEVPPSKEIKVWDSSSEMRFVVLPQRPAGTDGWSEEELATLVTRESMIGVEPAKAVA

SEQ ID NO: 31 - protein, 205 aa, Artificial
  Modified nitrile hydratase alpha-subunit
MTENILRKSDEEIQKEITARVKALESMLIEQGILTTSMIDRMAEIYEEEVGPHLGAKVVVKAWTDPEFKKRLLADGTEACKELGIGGLQGEDMMWVENTDEVHHVVVCTLCSCYPWPVLGLPPNWFKEPQYRSRVVREPRQLLKEEFGFEVPPSKEIKVWDSSSEMRFVVLPQRPAGTDGWSEEELATLVTRESMICVEPAKAVA

SEQ ID NO: 32 - protein, 205 aa, Artificial
  Modified nitrile hydratase alpha-subunit
MTENILRKSDEEIQKEITARVKALESMLIEQGILTSSMIDRMAEIYENEVGPHLGAKVVVKAWTDPEFKKRLLADGTEACKELGIGGLQGEEMMWVENTDEVHHVVVCTLCSCYPWPVLGLPPNWFKEPQYRSRVVREPRQLLKEEFGFEVPPSKEIKVWDSSSEMRFVVLPQRPAGTDGWSEEELATLVTRESMIGVEPAKAVA

SEQ ID NO: 33 - protein, 233 aa, Artificial
  Modified nitrile hydratase beta-subunit
MNGVYDVGGTDGLGPINRPADEPVFRAEWEKVAFAMFPATIRAGFMGLDEVRFGIEQMNPAEYLESPYYWHWIRTYIHHGVRTGKIDLEELERRTQYYRENPDAPLPDHEQKPELIEFVNQAVYGGLPASREVDRPPKFKEGDVVRFSTASPKGHARRARYVRGKTGTVVKHHGAYIYPDTAGNGLGECPEHLYTVRFTAQELWGPEGDPNSSVYYDCWEPYIELVDTKAAAA

SEQ ID NO: 34 - protein, 233 aa, Artificial
  Modified nitrile hydratase beta-subunit
MNGVYDVGGTDGLGPINRPADEPVFRAEWEKVAFAMFPATFRAGFKGLDEFRFGIEQMNPAEYLESPYYWHWIRTYIHHGVRTGKIDLEELERRTQYYRENPDAPLPRHEQKPELIEFVNQAVYGGLPASREVDRPPKFKEGDVVRFSTASPKGHARRARYVRGKTGTVVKHHGAYIYPDTAGNGLGECPEHLYTVRFTAQELWGPEGDPNYSVYYDCWEPYIELVDTKAAAA

SEQ ID NO: 35 - protein, 233 aa, Artificial
  Modified nitrile hydratase beta-subunit
MNGVYDVGGTDGLGPINRPADEPVFRAEWEKVAFAMFPATFRAGFMGLDEFRFGIEQMNPAEYLESPYYWHWIRTYIHHGVRTGKIDLEELERRTQYYRENPDAPLPEHEQKPELIEFVNQAVYGGSPASREVDRPPKFKEGDVVRFSTASPKGHARRAWYVRGKTGTVVKHHGAYIYPDTAGNGRGECPEHLYTVRFTAQELWGPEGDPNSSVYYDCWEPYIELVDTKAAAA

SEQ ID NO: 36 - protein, 233 aa, Artificial
  Modified nitrile hydratase beta-subunit
MNGMYDVGGTDGLGPINRPADEPVFRAEWEKVAFAMFPATFRAGFMGLDEFRFGIEQMNPAEYLESPYYWHWIRTYIHHGVRTGKIDLEELERRTQYYRENPDAPLPEHEQKPELIEFVNQAVYGGSPASREVDRPPKFKEGDVVRFSTASPKGHARRAWYVRGKTGTVVKHHGAYIYPDTAGNGRGECPEHLYTVRFTAQELWGPEGDPNSSVYYDCWEPYIELVDTKAAAA

SEQ ID NO: 37 - protein, 233 aa, Artificial
  Modified nitrile hydratase beta-subunit
MNGVYDVGGTDGLGPINRPADEPVFRAEWEKVAFAMLPATFRAGFMGLDEFRFGIEQMNPAEYLESPYYWHWIRTYIHHGVRTGKIDLEELERRTQYYRENPDAPLPDHEQKPELIEFVNQAVYGGLPASREVDRPPKFKEGDVVRFSTASPKGHARRARYVRGKTGTVVKHHGAYIYPDTAGNGLGECPEHLYTVRFTEQELWGPEGDPNSSVYYDCWEPYIELVDTKAAAA

SEQ ID NO: 38 - protein, 233 aa, Artificial
  Modified nitrile hydratase beta-subunit
MNGVYDVAGTDGLGPINRPADEPVFRAEWEKVAFAMLPATFRAGFMGLDEFRFGIEQMNPAEYLESPYYWHWIRTYIHHGVRTGKIDLEELERRTQYYRENPDAPLPDHEQKPELIEFVNQAVYGGLPASREVDRPPKFKEGDVVRFSTASPKGHARRARYVRGKTGTVVKHHGAYIYPDTAGNGLGECPEHLYTVRFTEQELWGPEGDPNSSVYYDCWEPYIELVDTKAAAA

SEQ ID NO: 39 - protein, 233 aa, Artificial
  Modified nitrile hydratase beta-subunit
MNGVYDVGGTDGLGPINRPADEPVFRAEWEKVAFAMVPATFRAGFMGLDEFRFGIEQMNPAEYLESPYYWHWIRTYIHHGVRTGKIDLEELERRTQYYRENPDAPLPDHEQKPELIEFVNQAVYGGLPASREVDRPPKFKEGDVVRFSTASPKGHARRARYVRGKTGTVVKHHGAYIYPDTAGNGLGECPEHLYTVRFTEQELWGPEGDPNSSVYYDCWEPYIELVDTKAAAA

SEQ ID NO: 40 - protein, 233 aa, Artificial
  Modified nitrile hydratase beta-subunit
MNGVYDVGGTDGLGPINRPADEPVFRAEWEKVAFAMVPATFRAGFMGLDEFRFGIEQMNPAEYLESPYYWHWIRTYIHNGVRTGKIDLEELERRTQYYRENPDAPLPDHEQKPELIEFVNQAVYGGLPASREVDRPPKFKEGDVVRFSTASPKGHARRARYVRGKTGTVVKHHGAYIYPDTAGNGLGECPEHLYTVRFTEQELWGPEGDPNSSVYYDCWEPYIELVDTKAAAA

SEQ ID NO: 41 - protein, 233 aa, Artificial
  Modified nitrile hydratase beta-subunit
MNGVYDVGGTDGLGPINRPADEPVFRAEWEKVAFAMFPATFRAGFMGVDEFRFGIEQMNPAEYLESPYYWHWIRTYIHHGVRTGKIDLEELERRTQYYRENPDAPLPRHEQKPELIEFVNQAVYGGLPASREVDRPPKFKEGDVVRFSTASPKGHARRARYVRGKTGTVVKHHGAYIYPDTAGNGLGECPEHLYTVRFTAQELWGPEGDPNYSVYYDCWEPYIELVDTKAAAA

SEQ ID NO: 42 - protein, 233 aa, Artificial
  Modified nitrile hydratase beta-subunit
MNGVYDVGGTDGLGPINRPADEPVFRAEWEKVAFAMFPATFRAGFMGVDEFRFGIEQMNPAEYLESPYYWHWIRTYIHHGVRTGKIDLEELERRTRYYRENPDAPLPRHEQKPELIEFVNQAVYGGLPASREVDRPPKFKEGDVVRFSTASPKGHARRARYVRGKTGTVVKHHGAYIYPDTAGNGLGECPEHLYTVRFTAQELWGPEGDPNYSVYYDCWEPYIELVDTKAAAA

SEQ ID NO: 43 - protein, 233 aa, Artificial
  Modified nitrile hydratase beta-subunit
MNGVYDVGGTDGLGPINRPADEPVFRAEWEKVAFAMVPATFRAGFMGLDEFRFGIEQMNPAEYLESPYYWHWIRTYIHHGVRTGKIDLEELERRTQYYRENPDAPLMDHEQKPELIEFVNQAVYGGLPASREVDRPPKFKEGDVVRFSTASPKGHARRARYVRGKTGTVVKHHGAYIYPDTAGNGLGECPEHLYTVRFTEQELWGPEGDPNSSVYYDCWEPYIELVDTKAAAA

SEQ ID NO: 44 - protein, 233 aa, Artificial
  Modified nitrile hydratase beta-subunit
MNGVYDVGGTDGLGPINRPADEPVFRAEWEKVAFAMLPATFRAGFMGLDEFRFGIEQMNPAEYLESPYYWHWIRTYIHHGVRTGKIDLEELERRTRYYRENPDAPLPDHEQKPELIEFVNQAVYGGLPASREVDRPPKFKEGDVVRFSTASPKGHARRARYVRGKTGTVVKHHGAYIYPDTAGNGLGECPEHLYTVRFTEQELWGPEGDPNSSVYYDCWEPYIELVDTKAAAA

SEQ ID NO: 45 - protein, 233 aa, Artificial
  Modified nitrile hydratase beta-subunit
MNGVYDVGGDDGLGPINRPADEPVFRAEWEKVAFAMFPATFRAGFMGLDEFRFGIEQMNPAEYLESPYYWHWIRTYIHHGVRTGKIDLEELERRTQYYRENPDAPLPEHEQKPELIEVVNQAVYGGLPASREVDRPPKFKEGDVVRFSTASPKGHARRARYVRGKTGTVVKHHGAYIYPDTAGNGLGECPEHLYTVRFTEQELWGPEGDPNSSVYYDCWEPYIELVDTKAAAA

SEQ ID NO: 46 - protein, 233 aa, Artificial
  Modified nitrile hydratase beta-subunit
MNGVYDVGGDDGLGPINRPADEPVFRAEWEKVAFAMFPATFRAGFMGLDEFRFGIEQMNPAEYLESPYYWHWIRTYIHHGVRTGKIDLEELERRTQYYRENPDAPLMEHEQKPELIEVVNQAVYGGLPASREVDRPPKFKEGDVVRFSTASPKGHARRARYVRGKTGTVVKHHGAYIYPDTAGNGLGECPEHLYTVRFTEQELWGPEGDPNSSVYYDCWEPYIELVDTKAAAA

SEQ ID NO: 47 - protein, 233 aa, Artificial
  Modified nitrile hydratase beta-subunit
MNGVYDVGGTDGLGPINRPADEPVFRAEWEKVAFAMFPATFRAGFMGLDEFRFGIEQMNPAEYLESPYYWHWIRTYIHHGVRTGKIDLEELERRTQYYRENPDAPLPDHEQKPELIEFVNQAVYGGLPASREVDRPPKFKEGDVVRFSTASPKGHARRARYVRGKTGTVVKHHGAYIYPDTAGNGLGECPEHLYTVRFTEQELWGPEGDPNSSVYYDCWEPYIELIDTKAAAA

SEQ ID NO: 48 - protein, 233 aa, Artificial
  Modified nitrile hydratase beta-subunit
MNGVYDVGGTDGLGPINRPADEPVFRAEWEKVAFAMFPATFRAGFMGVDEFRFGIEQMNPAEYLESPYYWHWIRTYIHNGVRTGKIDLEELERRTQYYRENPDAPLPRHEQKPELIEFVNQAVYGGLPASREVDRPPKFKEGDVVRFSTASPKGHARRARYVRGKTGTVVKHHGAYIYPDTAGNGLGECPEHLYTVRFTAQELWGPEGDPNYSVYYDCWEPYIELVDTKEAAA

SEQ ID NO: 49 - protein, 233 aa, Artificial
  Modified nitrile hydratase beta-subunit
MNGVYDVGGDDGLGPINRPADEPVFRAEWEKVAFAMFPATFRAGFMGLDEFRFGIEQMNPAEYLESPYYWHWIRTYIHHGVRTGKIDLEELERRTQYYRENPDAPLPEHEQKPELIEVVNQAVYGGLPASREVDRPPKFKEGDVVRFSTASPKGHARRARYVRGKTGTVVKHHGAYIYPDTAGNGLGECPEHLYTVRFTEQELWGLEGDPNSSVYYDCWEPYIELVDTKEAAA

SEQ ID NO: 50 - protein, 233 aa, Artificial
  Modified nitrile hydratase beta-subunit
MNGVYDVGGTDGLGPINRPADEPVFRAEWEKVAFAMFPATIRAGFMGLDEVRFGIEQMNPAEYLESPYYWHWIRTYIHHGVRTGKIDLEELERRTQYYRENPDAPLPDHEQKPELIEFVNQAVYGGLPASREVDRPPKFKEGDVVRFSTASPKGHARRARYVRGKTGTVVKHHGAYIYPDTAGNGLGECPEHLYTVRFTAQELWGLEGDPNSSVYYDCWEPYIELVDTKEAAA

SEQ ID NO: 51 - protein, 233 aa, Artificial
  Modified nitrile hydratase beta-subunit
MNGVYDVGGTDGLGPINRPADEPVFRAEWEKVAFAMFPATFRAGFMGLDEFRFGIEQMNPAEYLESPYYWHWIRTYIHHGVRTGKIDLEELERRTQYYRENPDAPLPEHNQKPELIEFVNQAVYGGLPASREVDRPPKFKEGDVVRFSTASPKGHARRARYVRGKTGTVVKHHGAYIYPDTAGNGLGECPEHLYTVRFTAQELWGPEGDPNSSVYYDCWEPYIELVDTKAAAA

SEQ ID NO: 52 - protein, 233 aa, Artificial
  Modified nitrile hydratase beta-subunit
MNGVYDVGGTDGLGPINRPADEPVFRAEWEKVAFAMFPATFRAGFKGLDEFRFGIEQMNPAEYLESPYYWHWIRTYIHHGVRTGKIDLEELERRTQYYRENPDAPLPRHNQKPELIEFVNQAVYGGLPASREVDRPPKFKEGDVVRFSTASPKGHARRARYVRGKTGTVVKHHGAYIYPDTAGNGLGECPEHLYTVRFTAQELWGPEGDPNYSVYYDCWEPYIELVDTKAAAA

SEQ ID NO: 53 - protein, 233 aa, Artificial
  Modified nitrile hydratase beta-subunit
MNGVYDVGGDDGLGPINRPADEPVFRAEWEKVAFAMFPATFRAGFMGLDEFRFGIEQMNPAEYLESPYYWHWIRTYIHHGVRTGKIDLEELERRTQYYRENPDAPLPEHEQKPELIEVVNQAVYGGLPASREVDRPPKFKEGDVVRFSTASPKGHARRARYVRGKTGTVVKHHGAYIYPDTAGNGLGECPEHLYTVRFTEQELWGLEGDPNSSVYYDCWEPYIELIDTKAAAA

SEQ ID NO: 54 - protein, 233 aa, Artificial
  Modified nitrile hydratase beta-subunit
MNGMYDVGGTDGLGPINRPADEPVFRAEWEKVAFAMFPATFRAGFMGLDEFRFGIEQMNPAEYLESPYYWHWIRTYIHHGVRTGKIDLEELERRTQYYRENPDAPLPEHEQKPELIEFVNQAVYGGLPASREVDRPPKFKEGDVVRFSTASPKGHARRARYVRGKTGTVVKHHGAYIYPDTAGNGLGECPEHLYTVRFTAQELWGLEGDPNSSVYYDCWEPYIELVDTKAAAA

SEQ ID NO: 55 - protein, 233 aa, Artificial
  Modified nitrile hydratase beta-subunit
MNGVYDVGGTDGLGPINRPADEPVFRAEWEKVAFAMFPATIRAGFMGLDEVRFGIEQMNPAEYLESPYYWHWIRTYIHHGVRTGKIDLEELERRTQYYRENPDAPLMDHEQKPELIEFVNQAVYGGLPASREVDRPPKFKEGDVVRFSTASPKGHARRARYVRGKTGTVVKHHGAYIYPDTAGNGLGECPEHLYTVRFTAQELWGPEGDPNSSVYYDCWEPYIELVDTKEAAA

SEQ ID NO: 56 - protein, 233 aa, Artificial
  Modified nitrile hydratase beta-subunit
MNGVYDVGGTDGLGPINRPADEPVFRAEWEKVAFAMFPATFRAGFMGVDEFRFGIEQMNPAEYLESPYYWHWIRTYIHNGVRTGKIDLEELERRTQYYRENPDAPLPRHEQKPELIEFVNQAVYGGLPASREVDRPPKFKEGDVVRFSTASPKGHARRARYVRGKTGTVVKHHGAYIYPDTAGNGLGECPEHLYTVRFTAQELWGPEGDPNYSVYYDCWEPYIELVDTKEVAA

SEQ ID NO: 57 - protein, 233 aa, Artificial
  Modified nitrile hydratase beta-subunit
MNGVYDVGGTDGLGPINRPADEPVFRAEWEKVAFAMFPATFRAGFKGLDEFRFGIEQMNPAEYLESPYYWHWIRTYIHNGVRTGKIDLEELERRTQYYRENPDAPLPRHEQKPELIEFVNQAVYGGLPASREVDRPPKFKEGDVVRFSTASPKGHARRARYVRGKTGTVVKHHGAYIYPDTAGNGLGECPEHLYTVRFTAQELWGPEGDPNYSVYYDCWEPYIELVDTKEVAA

SEQ ID NO: 58 - protein, 233 aa, Artificial
  Modified nitrile hydratase beta-subunit
MNGVYDVGGTDGLGPINRPADEPIFRAEWEKVAFAMFPATIRAGFMGLDEVRFGIEQMNPAEYLESPYYWHWIRTYIHHGVRTGKIDLEELERRTQYYRENPDAPLPDHEQKPELIEFVNQAVYGGLPASREVDRPPKFKEGDVVRFSTASPKGHARRARYVRGKTGTVVKHHGAYIYPDTAGNGLGECPEHLYTVRFTAQELWGPEGDPNSSVYYDCWEPYIELIDTKAAAA

SEQ ID NO: 59 - protein, 233 aa, Artificial
  Modified nitrile hydratase beta-subunit
MNGVYDVGGTDGLGPINRPADEPIFRAEWEKVAFAMFPATIRAGFMGLDEVRFGIEQMNPAEYLESPYYWHWIRTYIHHGVRTGKIDLEELERRTQYYRENPDAPLMDHEQKPELIEFVNQAVYGGLPASREVDRPPKFKEGDVVRFSTASPKGHARRARYVRGKTGTVVKHHGAYIYPDTAGNGLGECPEHLYTVRFTAQELWGPEGDPNSSVYYDCWEPYIELVDTKEAAA

SEQ ID NO: 60 - protein, 233 aa, Artificial
  Modified nitrile hydratase beta-subunit
MNGVYDVGGTDGLGPINRPADEPIFRAEWEKVAFAMFPATFRAGFMGLDEFRFGIEQMNPAEYLESPYYWHWIRTYIHHGVRTGKIDLEELERRTQYYRENPDAPLMEHEQKPELIEFVNQAVYGGLPASREVDRPPKFKEGDVVGFSTASPKGHARRARYVRGKTGTVVKHHGAYIYPDTAGNGLGECPEHLYTVRFTAQELWGPEGDPNSSVYYDCWEPYIELVDTKEAAA

SEQ ID NO: 61 - protein, 233 aa, Artificial
  Modified nitrile hydratase beta-subunit
MNGVYDVGGTDGLGPINRPADEPIFRAEWEKVAFAMFPATFRAGFMGVDEFRFGIEQMNPAEYLESPYYWHWIRTYIHNGVRTGKIDLEELERRTQYYRENPDAPLPRHEQKPELIEFVNQAVYGGLPASREVDRPPKFKEGDVVRFSTASPKGHARRARYVRGKTGTVVKHHGAYIYPDTAGNGLGECPEHLYTVRFTAQELWGPEGDPNYSVYYDCWEPYIELVDTKEVAA

SEQ ID NO: 62 - protein, 233 aa, Artificial
  Modified nitrile hydratase beta-subunit
MNGVYDVGGTDGLGPINRPADEPVFRAEWEKVVFAMFPATFRAGFMGLDEFRFGIEQMNPAEYLESPYYWHWIRTYIHHGVRTGKIDLEELERRTQYYRENPDAPLPEHEQKPELIEFVNQAVYGGLPASREVDRPPKFKEGDVVRFSTASPKGHARRARYVRGKTGTVVKHHGAYIYPDTAGNGLGECPEHLYTVRFTAQELWGPEGDPNSSVYYDCWEPYIELVDTKAAAA

SEQ ID NO: 63 - protein, 233 aa, Artificial
  Modified nitrile hydratase beta-subunit
MNGVYDVGGTDGLGPINRPADEPVFRAEWEKVAFAMFPAIFRAGFMGLDEFRFGIEQMNPVEYLESPYYWHWIRTYIHHGVRTGKIDLEELERRTQYYRENPDAPLPEHEQKPELIEFVNQAVYGGLPASREVDRPPKFKEGDVVRFSTASPKGHARRARYVRGKTGTVVKHHGAYIYPDTAGNGLGECPEHLYTVRFTAQELWGPEGDPNSSVYYDCWEPYIELVDTKAAAA

SEQ ID NO: 64 - protein, 233 aa, Artificial
  Modified nitrile hydratase beta-subunit
MNGVYDVGGTDGLGPINRPADEPVFRAEWEKVAFAMFPATIRAGFMGLDEVRFGIEQMNPAEYLESPYYWHWIRTYIHHGVRTGKIDLEELERRTQYYRENPDAPLPDHEQKPELIEFVNQAVYGGLPASREVDRPPKFKEGDVVRFSTASPKGHARRARYVRGKTGTVVKHHGAYIYPDTAGNGLGECPEHLYTVRFTAQELWGPEGDPNSSVYYDCWEPYIELIDTKAAAA

SEQ ID NO: 65 - protein, 233 aa, Artificial
  Modified nitrile hydratase beta-subunit
MNGVYDVGGTDGLGPINRPADEPVFRAEWEKVAFAMFPATFRAGFMGLDEFRFGIEQMNPLEYLESPYYWHWIRTYIHHGVRTGKIDLEELERRTQYYRENPDAPLPEHEQIPELIEFVNQAVYGGLPASREVDRPPKFKEGDVVRFSTASPKGHARRARYVRGKTGTVVKHHGAYIYPDTAGNGLGECPEHLYTVRFTAQELWGPEGDPNSSVYYDCWEPYIELIDTKAAAA

SEQ ID NO: 66 - protein, 233 aa, Artificial
  Modified nitrile hydratase beta-subunit
MNGMYDVGGTDGLGPINRPADEPVFRAEWEKVAFAMFPATFRAGFMGLDEVRFGIEQMNPAEYLESPYYWHWIRTYIHHGVRTGKIDLEELERRTQYYRENPDAPLPDHEQKPELIEFVNQAVYGGLPASREVDRPPKFKEGDVVRFSTASPKGHARRARYVRGKTGTVVKHHGAYIYPDTAGNGLGECPEHLYTVRFTAQELWGLEGDPNSSVYYDCWEPYIELVDTKAAAA

SEQ ID NO: 67 - protein, 233 aa, Artificial
  Modified nitrile hydratase beta-subunit
MNGVYDVGGTDGLGPINRPADEPVFRAEWEKVMFAMFPATFRAGFMGLDEFRFGIEQMNPAEYLESPYYWHWIRTYIHNGVRTGKIDLEELERRTQYYRENPDAPLPEHEQKPELIEFVNQAVYGGLPASREVDRPPKFKEGDVVRFSTASPKGHARRARYVRGKTGTVVKHHGATIYPDTAGNGLGECPEHLYTVRFTAQELWGPEGDPNSSVYYDCWEPYIELVDTKAAAA

SEQ ID NO: 68 - protein, 233 aa, Artificial
  Modified nitrile hydratase beta-subunit
MNGVYDVGGTDGLGPINRPADEPVFRAEWEKVAFAMFPATFRAGFMGLDEFRFGIEQMNPGEYLESPYYWHWIRTYIHNGVRTGKIDLEELERRTQYYRENPDAPLPEHEQKPELIEFVNQAVYGGLPASREVDRPPKFKEGDVVRFSTNSPKGHARRARYVRGKTGTVVKHHGAYIYPDTAGNGLGECPEHLYTVRFTAQELWGPEGDPNSSVYYDCWEPYIELVDTKAAAA

SEQ ID NO: 69 - protein, 233 aa, Artificial
  Modified nitrile hydratase beta-subunit
MNGMYDVGGTDGLGPINRPADEPVFRAEWEKVAFAMFPATFRAGFMGVDEFRFGIEQMNPAEYLESPYYWHWIRTYIHNGVRTGKIDLEELERRTQYYRENPDAPLPRHEQKPELIEFVNQAVYGGLPASREVDRPPKFKEGDVVRFSTASPKGHARRARYVRGKTGTVVKHHGAYIYPDTAGNGLGECPEHLYTVRFTAQELWGPEGDPNYSVYYDCWEPYIELVDTKAAAA

SEQ ID NO: 70 - protein, 233 aa, Artificial
  Modified nitrile hydratase beta-subunit
MNGMYDVGGTDGLGPINRPADEPVFRAEWEKVAFAMFPATFRAGFMGLDEFRFGIEQMNPTEYLESPYYWHWIRTYIHNGVRTGKIDLEELERRTQYYRENPDAPLPEHEQKPELIEFVNQAVYGGLPASREVDRPPKFKEGDVVRFSTASPKGHARRARYVRGKTGTVVKHHGAYIYPDTAGNGLGECPEHLYTVRFTAQELWGPEGDPNSSVYYDSWEPYIELVDTKAAAA

SEQ ID NO: 71 - protein, 233 aa, Artificial
  Modified nitrile hydratase beta-subunit
MNGMYDVGGTDGLGPINRPADEPVFRAEWEKVAFAMFPATFRAGFMGLDEFRFGIEQMNPAEYLESPYYWHWIRTYIHNGVRTGKIDLEELERRTQYYRENPDAPLPEHEQKPELIEFVNQAVYGGLPASREVDRPPKFKEGDVVGFSTASPKGHARRARYVRGKTGTVVKHHGAYIYPDTAGNGLGECPEHLYTVRFTAQELWGPEGDPNSSVYYSCWEPYIELVDTKAAAA

SEQ ID NO: 72 - protein, 233 aa, Artificial
  Modified nitrile hydratase beta-subunit
MNGVYDVGGTDGLGPINRPADEPVFRAEWEKVAFAMFPATFRAGFMGLDEFRFGIEQMNPAEYLESPYYWHWIRTYIHNGVRTGKIDLEELERRTQYYRENPDAPLPEHEQKPELIEFVNQAVYGGLPASREVDRPPKFKEGDVVRFSTASPKGHARRARYVRGKTGTVVKHHGAYIYPDTAGNGLGECPEHLYTVRFTAQELWGPEGDPNSSVYYDCWEPYIELVDTKEAAA

SEQ ID NO: 73 - protein, 233 aa, Artificial
  Modified nitrile hydratase beta-subunit
MNGVYDVGGDDGLGPINRPADEPVFRAEWEKVAFAMFPATFRAGFMGLDEFRFGIEQMNPAEYLESPYYWHWIRTYIHNGVRTGKIDLEELERRTQYYRENPDAPLPEHEQKPELIEVVNQAVYGGLPASREVDRPPKFKEGDVVRFSTASPKGHARRARYVRGKTGTVVKHHGAYIYPDTAGNGLGECPEHLYTVRFTEQELWGPEGDPNSSVYYDCWEPYIELVDTKEAAA

SEQ ID NO: 74 - DNA, 33 bp, Artificial
  Oligonucleotide to act as a PCR primer
tacgaattctaaggaggtctcagcatgaacggc

SEQ ID NO: 75 - protein, 144 aa, Pseudonocardia thermophila
MSAEAKVRLKHCPTAEDRAAADALLAQLPGGDRALDRGFDEPWQLRAFALAVAACRAGRFEWKQLQQALISSIGEWERTHDLDDPSWSYYEHFVAALESVLGEEGIVEPEALDERTAEVLANPPNKDHHGPHLEPVAVHPAVRS